European Patent Application EP 4 353 746 A1, published April 17, 2024. Title: ANTI-PD-1 HUMANIZED ANTIBODY OR ANTIGEN-BINDING FRAGMENT THEREOF AND APPLICATION THEREOF. Applicant: Guangdong Fapon Biopharma Inc. The sequence listing filed with the application follows.

SEQUENCE LISTING (15 sequences)

SEQ ID NO: 1 - DNA, 22 bp, Artificial Sequence
  Forward primer
ccgcaagcttgccgccaccatg

SEQ ID NO: 2 - DNA, 53 bp, Artificial Sequence
  Reverse primer
ccggaattctcattaatggtgatggtgatgatgctggaactggccggcaggtc

SEQ ID NO: 3 - protein, 120 aa, Artificial Sequence
  c22 VH
QVQLVQSGAEVKKPGASVKVSCKASGYTFTTYYMYWVRQAPGQGLEWMGGINPSNGGTNFNEKFKSRVTMTVDKSTSTAYMELSSLRSEDTAVYYCTRRDSNYDGGFDYWGQGTTVTVSS

SEQ ID NO: 4 - protein, 120 aa, Artificial Sequence
  c43 VH
QVQLVQSGAEVKKPGASVKVSCKASGYTFTTYYMYWVRQAPGQGLEWIGGINPSNGGTNYAEKFKGRVTLTVDTSTSTAYMELSSLRSEDTAVYYCTRRDSNYDGGFDYWGQGTTVTVSS

SEQ ID NO: 5 - protein, 120 aa, Artificial Sequence
  c53 VH
QVQLVQSGAEVKKPGASVKVSCKASGYTFTTYYMYWVRQAPGQGLEWMGGINPSNGGTNYAQKFQGRATMTVDTSTSTAYMELSSLRSEDTAVYYCTRRDSNYDGGFDYWGQGTTVTVSS

SEQ ID NO: 6 - protein, 112 aa, Artificial Sequence
  c22 VL
DIQLTQSPSSLSASVGDRATITCRASKSVSTSGYSYMHWYQQKPGKAPKLLIYLAYHLESGVPSRFSGSGSGTDFTLTISSVQPEDFATYYCQHSWELPITFGQGTKLEIKR

SEQ ID NO: 7 - protein, 112 aa, Artificial Sequence
  c43/c53 VL
DIQMTQSPSSLSASVGDRVTITCRASKSVSTSGYSYMHWYQQKPGKAPKLLIYLAYHLESGVPSRFSGSGSGTDFTLTISSLQPEDFATYYCQHSWELPITFGQGTKLEIKR

SEQ ID NO: 8 - protein, 5 aa, Artificial Sequence
  HCDR1
TYYMY

SEQ ID NO: 9 - protein, 17 aa, Artificial Sequence
  HCDR2
GINPSNGGTNFNEKFKS

SEQ ID NO: 10 - protein, 11 aa, Artificial Sequence
  HCDR3
RDSNYDGGFDY

SEQ ID NO: 11 - protein, 15 aa, Artificial Sequence
  LCDR1
RASKSVSTSGYSYMH

SEQ ID NO: 12 - protein, 7 aa, Artificial Sequence
  LCDR2
LAYHLES

SEQ ID NO: 13 - protein, 9 aa, Artificial Sequence
  LCDR3
QHSWELPIT

SEQ ID NO: 14 - protein, 120 aa, Artificial Sequence
  Heavy chain variable region
QVQLQQPGAELVKPGASVKLSCKASGYTFTTYYMYWVKQRPGQGLEWIGGINPSNGGTNFNEKFKSKATLTVDKSSSTAYMQLSSLTSEDSAVYYCTRRDSNYDGGFDYWGQGTTLTVSS

SEQ ID NO: 15 - protein, 112 aa, Artificial Sequence
  Light chain variable region
DIVLTQSPASLAVSLGQRATISCRASKSVSTSGYSYMHWYQQKPGQPPKLLIYLAYHLESGVPARFSGSGSGTDFTLNIHPVEEEDAATYYCQHSWELPITFGSGTKLEIKR